European Patent Application EP 4 215 042 A1, published July 26, 2023. Title: A non-human mammal comprising in its genome at least two human leukocyte antigen (HLA) class I alleles, methods of making such mammal and uses thereof. Applicant: T-Knife GmbH Max-Delbrueck-Centrum für Molekulare Medizin. The sequence listing filed with the application follows.

SEQUENCE LISTING (233 sequences)

SEQ ID NO: 1 - DNA, 24 bp, Artificial Sequence
  H-2DbFor-Primer
gtctggcgcgccttcttctacata

SEQ ID NO: 2 - DNA, 34 bp, Artificial Sequence
  H-2DbRev-Primer
ctcgcccttgctcaccatctgggatcccgggtgt

SEQ ID NO: 3 - DNA, 18 bp, Artificial Sequence
  eGFPFor-Primer
atggtgagcaagggcgag

SEQ ID NO: 4 - DNA, 35 bp, Artificial Sequence
  eGFPRev-Primer
gtctttaattaattacttgtacagctcgtccatgc

SEQ ID NO: 5 - DNA, 30 bp, Artificial Sequence
  CMV-Forward Primer_AscI
gctggcgcgccgtacgggccagatatacgc

SEQ ID NO: 6 - DNA, 31 bp, Artificial Sequence
  CMV-Reverse Primer_XmaI
gtccccggggtgggttctctagttagccaga

SEQ ID NO: 7 - DNA, 27 bp, Artificial Sequence
  For-H-2-Full-PA
atctgcatcctgtaagctccatgctac

SEQ ID NO: 8 - DNA, 37 bp, Artificial Sequence
  Rev-H-2-Full-PA
gtcttaattaaccatcacagatcaaaatggactgagc

SEQ ID NO: 9 - DNA, 37 bp, Artificial Sequence
  For-BGH-Full-PA
gactgctcttccaaactgtgccttctagttgccagcc

SEQ ID NO: 10 - DNA, 30 bp, Artificial Sequence
  Rev-BGH-Full-PA
gtcttaattaaccatagagcccaccgcatc

SEQ ID NO: 11 - DNA, 169 bp, Artificial Sequence
  Multiple cloning site (MCS) introduced into the pMA-V vector to clone six HLA alleles
ctatcgtaggcgcgcctccgatgcggccgcagttatcgcgcgcgattgtacgccggcgattgtacctgcaggcttaagattaccggtgccttgaagcttgttgcaggtacctcggcggagctcgaaggcgtactagtgctgatacgcgtcgtagctcgttaattaacgg

SEQ ID NO: 12 - DNA, 19 bp, Artificial Sequence
  MCS-FP
ctatcgtaggcgcgcctcc

SEQ ID NO: 13 - DNA, 24 bp, Artificial Sequence
  MCS-RP
ccgttaattaacgagctacgacgc

SEQ ID NO: 14 - DNA, 21 bp, Artificial Sequence
  FP-HLA-A3-AscI
cctaggcgcgccttcttctac

SEQ ID NO: 15 - DNA, 32 bp, Artificial Sequence
  RP-HLA-A3-NotI
agtacgcggccgcccatagagcccaccgcatc

SEQ ID NO: 16 - DNA, 37 bp, Artificial Sequence
  FP-HLA-A11-NotI
cgtagcggccgcgcgccttcttctacataaaacacac

SEQ ID NO: 17 - DNA, 33 bp, Artificial Sequence
  RP-HLA-A11-SbfI
cagttacctgcaggccatagagcccaccgcatc

SEQ ID NO: 18 - DNA, 37 bp, Artificial Sequence
  FP-HLA-B7-SbfI
cagccctgcagggccttcttctacataaaacacaccc

SEQ ID NO: 19 - DNA, 29 bp, Artificial Sequence
  RP-HLA-B7-AgeI
tgcaaccggtccatagagcccaccgcatc

SEQ ID NO: 20 - DNA, 37 bp, Artificial Sequence
  FP-HLA-B15-HindIII
ctagtgaagcttcgccttcttctacataaaacacacc

SEQ ID NO: 21 - DNA, 30 bp, Artificial Sequence
  RP-HLA-B15-KpnI
tcgacaggtacccatagagcccaccgcatc

SEQ ID NO: 22 - DNA, 34 bp, Artificial Sequence
  FP-HLA-C4-SacI
ctagagctccgccttcttctacataaaacacacc

SEQ ID NO: 23 - DNA, 28 bp, Artificial Sequence
  RP-HLA-C4-SpeI
gatactagtccatagagcccaccgcatc

SEQ ID NO: 24 - DNA, 35 bp, Artificial Sequence
  FP-HLA-C7-SpeI
tcagactagtcgccttcttctacataaaacacacc

SEQ ID NO: 25 - DNA, 31 bp, Artificial Sequence
  RP-HLA-C7-PacI
gacattaattaaccatagagcccaccgcatc

SEQ ID NO: 26 - protein, 9 aa, Artificial Sequence
  MAGE-A1 278
KVLEYVIKV

SEQ ID NO: 27 - protein, 9 aa, Artificial Sequence
  TRRAP nonamer (wild-type)
KLVFGSVSL

SEQ ID NO: 28 - protein, 50 aa, Artificial Sequence
  TRRAP_Homosap (Homo sapiens)
MGSNVELSNLYLKLFKLVFGSVSLFAAENEQMLKPHLHKIVNSSMELAQT

SEQ ID NO: 29 - protein, 50 aa, Artificial Sequence; identical to SEQ ID NO: 28
  TRRAP_Musmusc (Mus musculus)

SEQ ID NO: 30 - protein, 9 aa, Artificial Sequence
  TRRAP nonamer mutant epitope
KLVFGSVFL

SEQ ID NO: 31 - protein, 15 aa, Artificial Sequence
  TCR V-alpha chain, CDR3 region
CATDAEETSGSRLTF

SEQ ID NO: 32 - protein, 14 aa, Artificial Sequence
  TCR V-beta chain, CDR3 region
CASSLAGIYNEQFF

SEQ ID NO: 33 - protein, 14 aa, Artificial Sequence
  TCR V-alpha chain, CDR3 region
CAYRSPYSGAGSYQ

SEQ ID NO: 34 - protein, 14 aa, Artificial Sequence
  TCR V-alpha chain, CDR3 region
CILRDDSGNTPLVF

SEQ ID NO: 35 - protein, 14 aa, Artificial Sequence
  TCR V-beta chain, CDR3 region
CASSLAGAYNEQFF

SEQ ID NO: 36 - protein, 10 aa, Artificial Sequence
  Epitope
ASGAFGTVYK

SEQ ID NO: 37 - protein, 10 aa, Artificial Sequence
  Epitope
GSGAFGTVYK

SEQ ID NO: 38 - protein, 10 aa, Artificial Sequence
  Epitope
KTYTQSSHLK

SEQ ID NO: 39 - protein, 10 aa, Artificial Sequence
  Epitope
KTYTKSSHLK

SEQ ID NO: 40 - protein, 10 aa, Artificial Sequence
  Epitope
AISTRDPLSK

SEQ ID NO: 41 - protein, 10 aa, Artificial Sequence
  Epitope
AISTRDPLSE

SEQ ID NO: 42 - protein, 10 aa, Artificial Sequence
  Epitope
SLSFNNCFVK

SEQ ID NO: 43 - protein, 10 aa, Artificial Sequence
  Epitope
SLSFNDCFVK

SEQ ID NO: 44 - protein, 9 aa, Artificial Sequence
  Epitope
KVYEGVWKK

SEQ ID NO: 45 - protein, 9 aa, Artificial Sequence
  Epitope
EVYEGVWKK

SEQ ID NO: 46 - protein, 9 aa, Artificial Sequence
  Epitope
GLLKTVSYK

SEQ ID NO: 47 - protein, 9 aa, Artificial Sequence
  Epitope
ELLKTVSYK

SEQ ID NO: 48 - protein, 10 aa, Artificial Sequence
  Epitope
RVPHTNVVFK

SEQ ID NO: 49 - protein, 10 aa, Artificial Sequence
  Epitope
RVLHTNVVFK

SEQ ID NO: 50 - protein, 10 aa, Artificial Sequence
  Epitope
RMVRRAAASK

SEQ ID NO: 51 - protein, 10 aa, Artificial Sequence
  Epitope
PMVRRAAASK

SEQ ID NO: 52 - protein, 9 aa, Artificial Sequence
  Epitope
SSCMGSMNR

SEQ ID NO: 53 - protein, 9 aa, Artificial Sequence
  Epitope
SSCMGGMNR

SEQ ID NO: 54 - protein, 9 aa, Artificial Sequence
  Epitope
VVGAVGVGK

SEQ ID NO: 55 - protein, 9 aa, Artificial Sequence
  Epitope
VVGAGGVGK

SEQ ID NO: 56 - protein, 9 aa, Artificial Sequence
  Epitope
VVGAFGVGK

SEQ ID NO: 57 - protein, 9 aa, Artificial Sequence
  Epitope
VVGAGGVGK

SEQ ID NO: 58 - protein, 9 aa, Artificial Sequence
  Epitope
VVGASGVGK

SEQ ID NO: 59 - protein, 9 aa, Artificial Sequence
  Epitope
VVGAGGVGK

SEQ ID NO: 60 - protein, 9 aa, Artificial Sequence
  Epitope
VVGAGIVGK

SEQ ID NO: 61 - protein, 9 aa, Artificial Sequence
  Epitope
VVGAGGVGK

SEQ ID NO: 62 - protein, 10 aa, Artificial Sequence
  Epitope
ASGAFGTVYK

SEQ ID NO: 63 - protein, 10 aa, Artificial Sequence
  Epitope
GSGAFGTVYK

SEQ ID NO: 64 - protein, 10 aa, Artificial Sequence
  Epitope
TIESLPNLKK

SEQ ID NO: 65 - protein, 10 aa, Artificial Sequence
  Epitope
TIESLPNLKE

SEQ ID NO: 66 - protein, 10 aa, Artificial Sequence
  Epitope
KTYTQSSHLK

SEQ ID NO: 67 - protein, 10 aa, Artificial Sequence
  Epitope
KTYTKSSHLK

SEQ ID NO: 68 - protein, 9 aa, Artificial Sequence
  Epitope
KTVVNKLFK

SEQ ID NO: 69 - protein, 9 aa, Artificial Sequence
  Epitope
KTVVNKLFE

SEQ ID NO: 70 - protein, 10 aa, Artificial Sequence
  Epitope
TVCCMHLHEK

SEQ ID NO: 71 - protein, 10 aa, Artificial Sequence
  Epitope
TVRCMHLHEK

SEQ ID NO: 72 - protein, 9 aa, Artificial Sequence
  Epitope
TTAPPLSGK

SEQ ID NO: 73 - protein, 9 aa, Artificial Sequence
  Epitope
TTAPSLSGK

SEQ ID NO: 74 - protein, 9 aa, Artificial Sequence
  Epitope
TTAPALSGK

SEQ ID NO: 75 - protein, 9 aa, Artificial Sequence
  Epitope
TTAPSLSGK

SEQ ID NO: 76 - protein, 9 aa, Artificial Sequence
  Epitope
TTAPFLSGK

SEQ ID NO: 77 - protein, 9 aa, Artificial Sequence
  Epitope
TTAPSLSGK

SEQ ID NO: 78 - protein, 9 aa, Artificial Sequence
  Epitope
TTAPYLSGK

SEQ ID NO: 79 - protein, 9 aa, Artificial Sequence
  Epitope
TTAPSLSGK

SEQ ID NO: 80 - protein, 10 aa, Artificial Sequence
  Epitope
AISTRDPLSK

SEQ ID NO: 81 - protein, 10 aa, Artificial Sequence
  Epitope
AISTRDPLSE

SEQ ID NO: 82 - protein, 9 aa, Artificial Sequence
  Epitope
AMEVEEFLK

SEQ ID NO: 83 - protein, 9 aa, Artificial Sequence
  Epitope
TMEVEEFLK

SEQ ID NO: 84 - protein, 9 aa, Artificial Sequence
  Epitope
SSATEYLEK

SEQ ID NO: 85 - protein, 9 aa, Artificial Sequence
  Epitope
SSAMEYLEK

SEQ ID NO: 86 - protein, 10 aa, Artificial Sequence
  Epitope
MTTNGRLPVK

SEQ ID NO: 87 - protein, 10 aa, Artificial Sequence
  Epitope
KTTNGRLPVK

SEQ ID NO: 88 - protein, 9 aa, Artificial Sequence
  Epitope
GLLKTVSYK

SEQ ID NO: 89 - protein, 9 aa, Artificial Sequence
  Epitope
ELLKTVSYK

SEQ ID NO: 90 - protein, 10 aa, Artificial Sequence
  Epitope
RVPHTNVVFK

SEQ ID NO: 91 - protein, 10 aa, Artificial Sequence
  Epitope
RVLHTNVVFK

SEQ ID NO: 92 - protein, 10 aa, Artificial Sequence
  Epitope
ATLAGLVQYY

SEQ ID NO: 93 - protein, 10 aa, Artificial Sequence
  Epitope
ATLAELVQYY

SEQ ID NO: 94 - protein, 9 aa, Artificial Sequence
  Epitope
NPIFRFSSL

SEQ ID NO: 95 - protein, 9 aa, Artificial Sequence
  Epitope
DPIFRFSSL

SEQ ID NO: 96 - protein, 10 aa, Artificial Sequence
  Epitope
SPNGTIQNIL

SEQ ID NO: 97 - protein, 10 aa, Artificial Sequence
  Epitope
SPNGTIRNIL

SEQ ID NO: 98 - protein, 9 aa, Artificial Sequence
  Epitope
FPRELSRVL

SEQ ID NO: 99 - protein, 9 aa, Artificial Sequence
  Epitope
FLRELSRVL

SEQ ID NO: 100 - protein, 9 aa, Artificial Sequence
  Epitope
SPVLHTNVV

SEQ ID NO: 101 - protein, 9 aa, Artificial Sequence
  Epitope
SRVLHTNVV

SEQ ID NO: 102 - protein, 9 aa, Artificial Sequence
  Epitope
MVRSQRSAM

SEQ ID NO: 103 - protein, 9 aa, Artificial Sequence
  Epitope
MVRSQRSGM

SEQ ID NO: 104 - protein, 9 aa, Artificial Sequence
  Epitope
VPRFLTCNL

SEQ ID NO: 105 - protein, 9 aa, Artificial Sequence
  Epitope
VPRFLMCNL

SEQ ID NO: 106 - protein, 10 aa, Artificial Sequence
  Epitope
FQGEYIPTVF

SEQ ID NO: 107 - protein, 10 aa, Artificial Sequence
  Epitope
FPGEYIPTVF

SEQ ID NO: 108 - protein, 10 aa, Artificial Sequence
  Epitope
AQSYLYSSSY

SEQ ID NO: 109 - protein, 10 aa, Artificial Sequence
  Epitope
AQSYLYSGSY

SEQ ID NO: 110 - protein, 9 aa, Artificial Sequence
  Epitope
VLAPIGLVF

SEQ ID NO: 111 - protein, 9 aa, Artificial Sequence
  Epitope
VLAPIGLVL

SEQ ID NO: 112 - protein, 10 aa, Artificial Sequence
  Epitope
HSGATTTAPF

SEQ ID NO: 113 - protein, 10 aa, Artificial Sequence
  Epitope
HSGATTTAPS

SEQ ID NO: 114 - protein, 10 aa, Artificial Sequence
  Epitope
HSGATTTAPY

SEQ ID NO: 115 - protein, 10 aa, Artificial Sequence
  Epitope
HSGATTTAPS

SEQ ID NO: 116 - protein, 9 aa, Artificial Sequence
  Epitope
TQISSATEY

SEQ ID NO: 117 - protein, 9 aa, Artificial Sequence
  Epitope
TQISSAMEY

SEQ ID NO: 118 - protein, 10 aa, Artificial Sequence
  Epitope
VQKNEFISEF

SEQ ID NO: 119 - protein, 10 aa, Artificial Sequence
  Epitope
VQKNEFISEY

SEQ ID NO: 120 - protein, 9 aa, Artificial Sequence
  Epitope
YLCNACGFY

SEQ ID NO: 121 - protein, 9 aa, Artificial Sequence
  Epitope
YLCNACGLY

SEQ ID NO: 122 - protein, 10 aa, Artificial Sequence
  Epitope
IQNILGGTVF

SEQ ID NO: 123 - protein, 10 aa, Artificial Sequence
  Epitope
IRNILGGTVF

SEQ ID NO: 124 - protein, 10 aa, Artificial Sequence
  Epitope
FQSATDVAPF

SEQ ID NO: 125 - protein, 10 aa, Artificial Sequence
  Epitope
FQSATDVAAF

SEQ ID NO: 126 - protein, 10 aa, Artificial Sequence
  Epitope
RMAVLIFTEF

SEQ ID NO: 127 - protein, 10 aa, Artificial Sequence
  Epitope
RMAVLIFTDF

SEQ ID NO: 128 - protein, 10 aa, Artificial Sequence
  Epitope
RMAVLIFTHF

SEQ ID NO: 129 - protein, 10 aa, Artificial Sequence
  Epitope
RMAVLIFTDF

SEQ ID NO: 130 - protein, 9 aa, Artificial Sequence
  Epitope
YLDDRNTFL

SEQ ID NO: 131 - protein, 9 aa, Artificial Sequence
  Epitope
YLDDRNTFR

SEQ ID NO: 132 - protein, 10 aa, Artificial Sequence
  Epitope
SAPENPIFRF

SEQ ID NO: 133 - protein, 10 aa, Artificial Sequence
  Epitope
SAPEDPIFRF

SEQ ID NO: 134 - protein, 8 aa, Artificial Sequence
  Epitope
VFGSVFLF

SEQ ID NO: 135 - protein, 8 aa, Artificial Sequence
  Epitope
VFGSVSLF

SEQ ID NO: 136 - protein, 9 aa, Artificial Sequence
  Epitope
FSDAQRPSF

SEQ ID NO: 137 - protein, 9 aa, Artificial Sequence
  Epitope
FSDAQRPSS

SEQ ID NO: 138 - protein, 8 aa, Artificial Sequence
  Epitope
RFENGCYL

SEQ ID NO: 139 - protein, 8 aa, Artificial Sequence
  Epitope
MFENGCYL

SEQ ID NO: 140 - protein, 10 aa, Artificial Sequence
  Epitope
IVDGAVFAVF

SEQ ID NO: 141 - protein, 10 aa, Artificial Sequence
  Epitope
IVDGAVFAVL

SEQ ID NO: 142 - protein, 8 aa, Artificial Sequence
  Epitope
FYIITELM

SEQ ID NO: 143 - protein, 8 aa, Artificial Sequence
  Epitope
FYIITEFM

SEQ ID NO: 144 - protein, 10 aa, Artificial Sequence
  Epitope
YTDVSNMSHL

SEQ ID NO: 145 - protein, 10 aa, Artificial Sequence
  Epitope
YTDVSNMSRL

SEQ ID NO: 146 - protein, 10 aa, Artificial Sequence
  Epitope
YTDVSNMSCL

SEQ ID NO: 147 - protein, 10 aa, Artificial Sequence
  Epitope
YTDVSNMSRL

SEQ ID NO: 148 - protein, 10 aa, Artificial Sequence
  Epitope
RYIMSDSNYV

SEQ ID NO: 149 - protein, 10 aa, Artificial Sequence
  Epitope
RDIMSDSNYV

SEQ ID NO: 150 - protein, 9 aa, Artificial Sequence
  Epitope
MYDKEYDSV

SEQ ID NO: 151 - protein, 9 aa, Artificial Sequence
  Epitope
MYDKEYYSV

SEQ ID NO: 152 - protein, 11 aa, Artificial Sequence
  Epitope
VYPEIDNRQCV

SEQ ID NO: 153 - protein, 11 aa, Artificial Sequence
  Epitope
VYLEIDNRQCV

SEQ ID NO: 154 - protein, 11 aa, Artificial Sequence
  Epitope
YYDLYGGEKFV

SEQ ID NO: 155 - protein, 11 aa, Artificial Sequence
  Epitope
YYDLYGGEKFA

SEQ ID NO: 156 - protein, 9 aa, Artificial Sequence
  Epitope
SYLGVAEAL

SEQ ID NO: 157 - protein, 9 aa, Artificial Sequence
  Epitope
SDLGVAEAL

SEQ ID NO: 158 - protein, 10 aa, Artificial Sequence
  Epitope
FVLAPIGLVF

SEQ ID NO: 159 - protein, 10 aa, Artificial Sequence
  Epitope
FVLAPIGLVL

SEQ ID NO: 160 - protein, 10 aa, Artificial Sequence
  Epitope
FAVFKAVFVL

SEQ ID NO: 161 - protein, 10 aa, Artificial Sequence
  Epitope
FAVLKAVFVL

SEQ ID NO: 162 - protein, 9 aa, Artificial Sequence
  Epitope
LAARNILVF

SEQ ID NO: 163 - protein, 9 aa, Artificial Sequence
  Epitope
LAARNILVA

SEQ ID NO: 164 - protein, 9 aa, Artificial Sequence
  Epitope
RFLTCNLAF

SEQ ID NO: 165 - protein, 9 aa, Artificial Sequence
  Epitope
RFLMCNLAF

SEQ ID NO: 166 - protein, 10 aa, Artificial Sequence
  Epitope
RMAVLIFTEF

SEQ ID NO: 167 - protein, 10 aa, Artificial Sequence
  Epitope
RMAVLIFTDF

SEQ ID NO: 168 - protein, 11 aa, Artificial Sequence
  Epitope
YTHSEYYNHAF

SEQ ID NO: 169 - protein, 11 aa, Artificial Sequence
  Epitope
YTHSEYYNHAI

SEQ ID NO: 170 - protein, 10 aa, Artificial Sequence
  Epitope
YAKVSTCLPM

SEQ ID NO: 171 - protein, 10 aa, Artificial Sequence
  Epitope
YAKVSICLPM

SEQ ID NO: 172 - protein, 13 aa, Artificial Sequence
  NY- ESO peptide
APRGPHGGAASGL

SEQ ID NO: 173 - protein, 9 aa, Artificial Sequence
  mutated calreticulin (mCALR) protein-derived epitope
KMRMRRMRR

SEQ ID NO: 174 - protein, 9 aa, Artificial Sequence
  mutated KRAS protein-derived G12V epitope
VVGAVGVGK

SEQ ID NO: 175 - protein, 10 aa, Artificial Sequence
  CMV epitope
TPRVTGGGAM

SEQ ID NO: 176 - protein, 9 aa, Artificial Sequence
  HPV epitope
SAFRCFIVY

SEQ ID NO: 177 - protein, 9 aa, Artificial Sequence
  CMV epitope
QYDPVAALF

SEQ ID NO: 178 - protein, 9 aa, Artificial Sequence
  MAGE-A12 epitope
VRIGHLYIL

SEQ ID NO: 179 - protein, 9 aa, Artificial Sequence
  MAGE-A1 epitope
KVLEYVIKV

SEQ ID NO: 180 - protein, 13 aa, Artificial Sequence
  NY- ESO epitope
APRGPHGGAASGL

SEQ ID NO: 181 - protein, 14 aa, Artificial Sequence
  CDR3 region
CALSDRERDDKIIF

SEQ ID NO: 182 - protein, 13 aa, Artificial Sequence
  CDR3 region
CASSHEGLAGEFF

SEQ ID NO: 183 - protein, 9 aa, Artificial Sequence
  Epitope
KMRMRRMRR

SEQ ID NO: 184 - protein, 16 aa, Artificial Sequence
  CDR3 region
CAVSGGTNSAGNKLTF

SEQ ID NO: 185 - protein, 14 aa, Artificial Sequence
  CDR3 region
CASSRDWGPAEQFF

SEQ ID NO: 186 - protein, 9 aa, Artificial Sequence
  Epitope
VVGAVGVGK

SEQ ID NO: 187 - protein, 15 aa, Artificial Sequence
  CDR3 region
CATVIRMDSSYKLIF

SEQ ID NO: 188 - protein, 16 aa, Artificial Sequence
  CDR3 region
CASSLIGVSSYNEQFF

SEQ ID NO: 189 - protein, 10 aa, Artificial Sequence
  Epitope
TPRVTGGGAM

SEQ ID NO: 190 - protein, 12 aa, Artificial Sequence
  CDR3 region
CAESEYGNKLVF

SEQ ID NO: 191 - protein, 13 aa, Artificial Sequence
  CDR3 region
CASSYRQQETQYF

SEQ ID NO: 192 - protein, 9 aa, Artificial Sequence
  Epitope
SAFRCFIVY

SEQ ID NO: 193 - protein, 13 aa, Artificial Sequence
  CDR3 region
CILRDNTGNQFYF

SEQ ID NO: 194 - protein, 15 aa, Artificial Sequence
  CDR3 region
CATSRDGSSYNEQFF

SEQ ID NO: 195 - protein, 9 aa, Artificial Sequence
  Epitope
QYDPVAALF

SEQ ID NO: 196 - protein, 12 aa, Artificial Sequence
  CDR3 region
CAASGATDKLIF

SEQ ID NO: 197 - protein, 11 aa, Artificial Sequence
  CDR3 region
CASSGGHEQYF

SEQ ID NO: 198 - protein, 9 aa, Artificial Sequence
  Epitope
VRIGHLYIL

SEQ ID NO: 199 - protein, 9 aa, Artificial Sequence
  dominant HLA-A*02-restricted MAGE-A1 epitope
KVLEYVIKV

SEQ ID NO: 200 - protein, 9 aa, Artificial Sequence
  MAGE-A1 epitope
GTLEEVPTA

SEQ ID NO: 201 - protein, 9 aa, Artificial Sequence
  Predicted nonamer binder
SLHCKPEEA

SEQ ID NO: 202 - protein, 9 aa, Artificial Sequence
  Predicted nonamer binder
AQQEALGLV

SEQ ID NO: 203 - protein, 9 aa, Artificial Sequence
  Predicted nonamer binder
ALGLVCVQA

SEQ ID NO: 204 - protein, 9 aa, Artificial Sequence
  Predicted nonamer binder
GLVCVQAAT

SEQ ID NO: 205 - protein, 9 aa, Artificial Sequence
  Predicted nonamer binder
ATSSSSPLV

SEQ ID NO: 206 - protein, 9 aa, Artificial Sequence
  Predicted nonamer binder
STSCILESL

SEQ ID NO: 207 - protein, 9 aa, Artificial Sequence
  Predicted nonamer binder
KVLEYVIKV

SEQ ID NO: 208 - DNA, 15073 bp, Artificial Sequence
  DNA sequence of the ABab.I transgene construct in the founder mice
gcaggctgaataataaaaaaattagaaactattatttaaccctagaaagataatcatattgtgacgtacgttaaagataatcatgcgtaaaattgacgcatgtgttttatcggtctgtatatcgaggtttatttattaatttgaatagatattaagttttattatatttacacttacatactaataataaattcaacaaacaatttatttatgtttatttatttattaaaaaaaaacaaaaactcaaaatttcttctataaagtaacaaaacttttaaacattctctcttttacaaaaataaacggcgcgccttcttctacataaaacacacccatctggagctacagaggcttcatatgggaagaaacaggaggagtctgagactaagcccgaggctgagaagacagatcctgaggaaataggcaaagtctcccctttacagatgagagtcctgcactcaggcttggcagtgtgagccgcccattgcaggtgaacagagcctggtctctgtgggatccctgtggggcttgcaggccagcgcctctgctttaaagagaagcctctctccactgcatccctaagcgcttgtgtcgccattgtattcccggaagtgacctttcttctagaagactctagggtgtgacttctgaagagaagaaggaagaggaagggtggaggttaggaaacagtgagtcgggcttgtgggtctctcctggtgatctgacagcttctgggtcagaactcggagtcaccacgacaaactgctctctgtccgcagtacagggttcaggcaaagtcttggttgccaggcggtgaggtcaggggtggggaagcccagggctggggattccccatctcctcagtttcacttctgcacctaacctgggtcaggtccttctgccgggacactgatgacgcgctggcaggtctcactatcattgggtggcgagattccaggagccaatcagcgtcgccgcggacgctggttataaagtccacgcaacccgcgggactcagacacccgggatcccagatgggcgccatggcccctagaaccctgctgctgctcctggccgctgccctggcccctacccagaccagagccatccagagaacccccaagatccaggtgtacagcagacaccccgccgagaacggcaagagcaacttcctgaactgctacgtgtccggcttccaccccagcgacatcgaggtggacctgctgaagaacggcgagagaatcgagaaggtggaacacagcgacctgagcttcagcaaggactggtccttctacctgctgtactacaccgagttcacccccaccgagaaggacgagtacgcctgcagagtgaaccacgtgaccctgagccagcccaagatcgtgaagtgggacagagacatgggcggaggcggctctggtggcggaggaagcggaggcggaggcagcggcagccacagcatgagatactttttcaccagcgtgtccagacccggcagaggcgagcccagattcattgccgtgggctacgtggacgacacccagttcgtcagattcgacagcgacgccgccagccagagaatggaacccagagccccctggatcgagcaggaaggccccgagtactgggaccaggaaaccagaaacgtcaaggcccagagccagaccgacagagtggacctgggcaccctgagaggctactacaaccagagcgaggccggctcccacaccatccagattatgtacggctgcgacgtgggcagcgacggcagattcctgaggggctacagacaggacgcctacgacggcaaggactatatcgccctgaacgaggacctgagaagctggacagccgccgacatggccgcccagatcaccaagagaaagtgggaggccgcccacgaggccgagcagctgagagcctacctggacggcacctgtgtggaatggctgcggagatacctggaaaacggcaaagagacactgcagagaaccgacagccccaaggcccacgtgacacaccaccctagaagcaagggcgaagtgaccctgcggtgctgggctctgggcttctaccccgccgacatcaccctgacctggcagctgaacggcgaggaactgacccaggacatggaactggtggaaaccagacctgccggcgacggcaccttccagaaatgggccagcgtggtggtgcccctgggcaaagagcagaactacacctgtagagtgtaccacgagggcctgcccgagcccctgaccctgagatgggagcctcctcccagcaccgactcctacatggtcatcgtggccgtgctgggagtgctgggcgctatggccatcatcggcgccgtggtggccttcgtgatgaagaggcggagaaacaccggcggcaagggcggcgattacgccctggctcctggcagccagagcagcgagatgagcctgagagactgcaaggcctgactgtgccttctagttgccagccatctgttgtttgcccctcccccgtgccttccttgaccctggaaggtgccactcccactgtcctttcctaataaaatgaggaaattgcatcgcattgtctgagtaggtgtcattctattctggggggtggggtggggcaggacagcaagggggaggattgggaagacaatagcaggcatgctggggatgcggtgggctctatgggcggccgcgcgccttcttctacataaaacacacccatctggagctacagaggcttcatatgggaagaaacaggaggagtctgagactaagcccgaggctgagaagacagatcctgaggaaataggcaaagtctcccctttacagatgagagtcctgcactcaggcttggcagtgtgagccgcccattgcaggtgaacagagcctggtctctgtgggatccctgtggggcttgcaggccagcgcctctgctttaaagagaagcctctctccactgcatccctaagcgcttgtgtcgccattgtattcccggaagtgacctttcttctagaagactctagggtgtgacttctgaagagaagaaggaagaggaagggtggaggttaggaaacagtgagtcgggcttgtgggtctctcctggtgatctgacagcttctgggtcagaactcggagtcaccacgacaaactgctctctgtccgcagtacagggttcaggcaaagtcttggttgccaggcggtgaggtcaggggtggggaagcccagggctggggattccccatctcctcagtttcacttctgcacctaacctgggtcaggtccttctgccgggacactgatgacgcgctggcaggtctcactatcattgggtggcgagattccaggagccaatcagcgtcgccgcggacgctggttataaagtccacgcaacccgcgggactcagacacccgggatcccagatgggcgccatggcccctagaaccctgctgctgctcctggccgctgccctggcccctacccagaccagagccatccagagaacccccaagatccaggtgtacagcagacaccccgccgagaacggcaagagcaacttcctgaactgctacgtgtccggcttccaccccagcgacatcgaggtggacctgctgaagaacggcgagagaatcgagaaggtggaacacagcgacctgagcttcagcaaggactggtccttctacctgctgtactacaccgagttcacccccaccgagaaggacgagtacgcctgcagagtgaaccacgtgaccctgagccagcccaagatcgtgaagtgggacagagacatgggcggaggcggctctggtggcggaggaagcggaggcggaggcagcggcagccacagcatgagatacttttacacctccgtgtcccggcctggcaggggagagcctcggtttatcgccgtgggatatgtggatgatacacagtttgtccgcttcgactccgacgccgcctctcagcggatggaacctcgggctccctggattgaacaggaaggacctgaatattgggatcaggaaacacggaacgtcaaagctcagtcccagacagaccgggtcgacctgggaacactgcggggatattacaaccagtccgaggatggcagccatacaattcagattatgtatggatgtgatgtgggccctgacggccggttcctgagaggataccggcaggatgcttacgatggaaaggattacattgccctcaatgaggacctgcggtcctggaccgccgctgatatggctgctcagattacaaagcggaagtgggaagctgctcacgccgctgagcagcagcgggcttacctggaaggcagatgcgtcgagtggctgaggcgctacctcgagaacggaaaagaaaccctgcagcggaccgactctcctaaggctcacgtgacccatcatcccaggtccaagggggaagtcacactgagatgttgggccctgggcttttatcctgctgatattaccctcacatggcagctcaatggggaagaactcacacaggatatggaactcgtcgagacaaggcccgctggcgacggaacatttcagaagtgggcttccgtcgtcgtgcctctcggaaaagaacagaattacacatgccgggtgtaccatgaaggactgcctgaacctctcacactccgctgggagcccccaccctccacagacagctatatggtcattgtcgctgtgctcggcgtcctgggagccatggctatcattggagctgtggtcgcttttgtcatgaagcgcagaagaaacacagggggaaaaggcggagactacgctctggccccaggctcccagtccagcgagatgtctctgcgggattgcaaggcttgactgtgccttctagttgccagccatctgttgtttgcccctcccccgtgccttccttgaccctggaaggtgccactcccactgtcctttcctaataaaatgaggaaattgcatcgcattgtctgagtaggtgtcattctattctggggggtggggtggggcaggacagcaagggggaggattgggaagacaatagcaggcatgctggggatgcggtgggctctatggcctgcagggccttcttctacataaaacacacccatctggagctacagaggcttcatatgggaagaaacaggaggagtctgagactaagcccgaggctgagaagacagatcctgaggaaataggcaaagtctcccctttacagatgagagtcctgcactcaggcttggcagtgtgagccgcccattgcaggtgaacagagcctggtctctgtgggatccctgtggggcttgcaggccagcgcctctgctttaaagagaagcctctctccactgcatccctaagcgcttgtgtcgccattgtattcccggaagtgacctttcttctagaagactctagggtgtgacttctgaagagaagaaggaagaggaagggtggaggttaggaaacagtgagtcgggcttgtgggtctctcctggtgatctgacagcttctgggtcagaactcggagtcaccacgacaaactgctctctgtccgcagtacagggttcaggcaaagtcttggttgccaggcggtgaggtcaggggtggggaagcccagggctggggattccccatctcctcagtttcacttctgcacctaacctgggtcaggtccttctgccgggacactgatgacgcgctggcaggtctcactatcattgggtggcgagattccaggagccaatcagcgtcgccgcggacgctggttataaagtccacgcaacccgcgggactcagacacccgggatcccagatgggcgccatggcccctagaaccctgctgctgctcctggccgctgccctggcccctacccagaccagagccatccagcgcactcctaagattcaggtctacagccgccacccagctgaaaacggaaagtccaatttcctcaactgctatgtctctggatttcacccctccgacattgaagtggacctgctcaaaaatggcgaacgcattgagaaagtcgagcatagcgatctcagcttctccaaggattggtctttttatctgctctattacacagaattcacccctacagaaaaggatgaatacgcatgtcgagtgaatcacgtcacactctcccagccaaaaattgtgaagtgggaccgcgatatgggaggcggaggatctgggggaggtggtagcggagggggcggatccggctctcactccatgagatatttctacacatctgtgtctaggcccggacggggcgagccccggttcatctctgtcggatacgtcgacgatactcagtttgtcagatttgactctgatgccgctagccccagagaggaaccacgcgccccttggatcgaacaggaagggccagagtattgggaccggaacacccagatctacaaggctcaggcccagaccgatcgcgagagcctgagaaacctgagggggtactacaatcagtccgaagccggaagccacaccctgcagtctatgtacggttgtgacgtcggccccgatggcagactgctgagaggccacgaccagtacgcttatgacggcaaagactacattgctctcaacgaagatctccgcagctggaccgctgccgataccgctgcacagatcacccagcgcaaatgggaagccgctagagaggctgagcagagaagggcctacctcgagggcgagtgtgtcgaatggctcagacggtatctggaaaatggcaaggacaagctggaaagggccgactcccccaaagcacatgtgacccaccatccacgcagcaaaggcgaagtcactctccgctgttgggcactcggattctacccagctgatattacactgacttggcagctgaatggggaggaactgactcaggatatggaactggtcgagactcgcccagccggggatggaacttttcagaaatgggcctctgtggtcgtcccactgggaaaagagcagaattatacctgtcgcgtctaccatgagggactcccagagccactcactctcagatgggaaccccccccatctaccgatagttacatggtcattgtggcagtcctcggggtgctcggtgccatggccattatcggggctgtcgtggcatttgtcatgaagagaaggcgcaacacaggcgggaaggggggggactatgcactggcccctggaagccagtcctccgagatgagtctccgggactgtaaagcctgactgtgccttctagttgccagccatctgttgtttgcccctcccccgtgccttccttgaccctggaaggtgccactcccactgtcctttcctaataaaatgaggaaattgcatcgcattgtctgagtaggtgtcattctattctggggggtggggtggggcaggacagcaagggggaggattgggaagacaatagcaggcatgctggggatgcggtgggctctatggaccggtgccttgaagcttcgccttcttctacataaaacacacccatctggagctacagaggcttcatatgggaagaaacaggaggagtctgagactaagcccgaggctgagaagacagatcctgaggaaataggcaaagtctcccctttacagatgagagtcctgcactcaggcttggcagtgtgagccgcccattgcaggtgaacagagcctggtctctgtgggatccctgtggggcttgcaggccagcgcctctgctttaaagagaagcctctctccactgcatccctaagcgcttgtgtcgccattgtattcccggaagtgacctttcttctagaagactctagggtgtgacttctgaagagaagaaggaagaggaagggtggaggttaggaaacagtgagtcgggcttgtgggtctctcctggtgatctgacagcttctgggtcagaactcggagtcaccacgacaaactgctctctgtccgcagtacagggttcaggcaaagtcttggttgccaggcggtgaggtcaggggtggggaagcccagggctggggattccccatctcctcagtttcacttctgcacctaacctgggtcaggtccttctgccgggacactgatgacgcgctggcaggtctcactatcattgggtggcgagattccaggagccaatcagcgtcgccgcggacgctggttataaagtccacgcaacccgcgggactcagacacccgggatcccagatgggcgccatggcccctagaaccctgctgctgctcctggccgctgccctggcccctacccagaccagagccattcagaggactccaaaaatccaggtctactctagacatcctgccgaaaatgggaaaagcaattttctgaattgctacgtcagcgggttccacccatctgacattgaggtcgacctgctcaagaacggggaacggattgaaaaggtggaacattctgacctgagcttttctaaagattggtccttctatctcctgtattatactgaattcactccaaccgaaaaagacgaatatgcatgccgcgtgaaccatgtcactctgtctcagcccaaaatcgtcaagtgggatcgggatatgggcggagggggttctggcggtggtggatctggcgggggaggttccggcagccactccatgcgctacttttacacagccatgagcaggcccggcaggggggaaccacggttcattgcagtcggctatgtcgacgatacacagttcgtccgctttgatagcgacgccgcttcccccagaatggcccccagggcaccttggattgagcaggaaggtccagaatactgggatcgcgagacacagatcagcaagaccaacacccagacatacagagagtccctgcgcaacctgcgcggctactataatcagtctgaggctggctcccataccctgcagaggatgtatggatgcgacgtcggaccagacggccggctgctgaggggacacgatcagagcgcctatgatggaaaagattatatcgctctgaatgaagatctgtcctcttggaccgcagccgacacagcagcccagattactcagcgcaagtgggaggcagccagggaagccgagcagtggcgggcctatctggaaggactgtgcgtggaatggctgcgccggtatctcgagaatgggaaagagactctccagcgcgccgattcccctaaggcccatgtcacacatcatccaagatctaaaggcgaagtgacactcagatgctgggcactcggtttttatccagcagacatcactctcacttggcagctgaatggcgaagaactcactcaggacatggaactggtcgaaacacggccagctggggacgggacattccagaaatgggcatctgtcgtggtgcctctggggaaagaacagaactatacttgccgagtctatcacgaagggctgccagaacctctgactctcagatgggagccaccacctagcacagatagttatatggtcatcgtcgccgtcctgggtgtcctcggggcaatggcaattattggcgccgtggtcgcatttgtgatgaagcggaggcggaataccggcggaaagggtggcgactatgctctcgctcccggatctcagagttccgagatgtccctcagggactgcaaagcatgactgtgccttctagttgccagccatctgttgtttgcccctcccccgtgccttccttgaccctggaaggtgccactcccactgtcctttcctaataaaatgaggaaattgcatcgcattgtctgagtaggtgtcattctattctggggggtggggtggggcaggacagcaagggggaggattgggaagacaatagcaggcatgctggggatgcggtgggctctatgggtacctcggcggagctccgccttcttctacataaaacacacccatctggagctacagaggcttcatatgggaagaaacaggaggagtctgagactaagcccgaggctgagaagacagatcctgaggaaataggcaaagtctcccctttacagatgagagtcctgcactcaggcttggcagtgtgagccgcccattgcaggtgaacagagcctggtctctgtgggatccctgtggggcttgcaggccagcgcctctgctttaaagagaagcctctctccactgcatccctaagcgcttgtgtcgccattgtattcccggaagtgacctttcttctagaagactctagggtgtgacttctgaagagaagaaggaagaggaagggtggaggttaggaaacagtgagtcgggcttgtgggtctctcctggtgatctgacagcttctgggtcagaactcggagtcaccacgacaaactgctctctgtccgcagtacagggttcaggcaaagtcttggttgccaggcggtgaggtcaggggtggggaagcccagggctggggattccccatctcctcagtttcacttctgcacctaacctgggtcaggtccttctgccgggacactgatgacgcgctggcaggtctcactatcattgggtggcgagattccaggagccaatcagcgtcgccgcggacgctggttataaagtccacgcaacccgcgggactcagacacccgggatcccagatgggcgccatggcccctagaaccctgctgctgctcctggccgctgccctggcccctacccagaccagagccattcagcgcacacctaagatccaggtgtactctcggcatcccgccgagaacgggaagtctaatttcctcaattgctacgtgtcagggttccatccatccgacatcgaagtggatctgctcaagaacggggaaaggatcgagaaagtcgaacacagtgatctgtcattctctaaagactggtctttctacctcctctattacactgagttcacacctactgagaaagatgaatacgcctgccgggtcaaccacgtcacactcagtcagccaaagatcgtgaaatgggatagggatatgggtggcggaggctccggcggaggcggatcagggggaggcggatctggcagccattctatgagatacttcagcacaagcgtgtcctggccagggcgaggcgagccacgctttattgcagtgggttatgtcgatgacacccagtttgtccgatttgattcagacgctgccagccccaggggcgagcctagagaaccttgggtggaacaggaaggtcctgagtactgggatagagaaacccagaagtacaagagacaggcccaggctgatagagtgaacctgagaaagctgcgcgggtattataaccagagtgaagatggctctcacaccctccagcggatgttcggctgtgacctgggcccagacggtagactgctgcggggctacaaccagttcgcctatgacgggaaggattacattgcactgaacgaggatctgagatcttggaccgccgcagacaccgccgctcagattacccagaggaaatgggaggctgctcgcgaagccgaacagcgcagagcctatctcgagggaacctgcgtcgaatggctgagaagatatctcgagaacggcaaagaaacactccagagggctgactctccaaaagctcatgtcactcaccacccccgctctaagggggaagtgactctcaggtgttgggctctggggttttacccagcagatatcactctgacctggcagctcaacggggaagaactcacccaggacatggaactcgtggaaactcggcccgcaggcgacgggacttttcagaaatgggcaagcgtcgtcgtgccactcggcaaagagcagaactatacttgcagggtctaccatgagggcctgcctgaaccactgacactccgatgggaaccacctccttcaaccgactcttatatggtcattgtggctgtcctgggcgtgctgggggctatggctattattggtgcagtcgtggctttcgtcatgaagcggcgacggaatactgggggcaaggggggagactacgccctcgcacctggttctcagtcctctgaaatgtctctccgcgactgcaaagcttgactgtgccttctagttgccagccatctgttgtttgcccctcccccgtgccttccttgaccctggaaggtgccactcccactgtcctttcctaataaaatgaggaaattgcatcgcattgtctgagtaggtgtcattctattctggggggtggggtggggcaggacagcaagggggaggattgggaagacaatagcaggcatgctggggatgcggtgggctctatggactagtcgccttcttctacataaaacacacccatctggagctacagaggcttcatatgggaagaaacaggaggagtctgagactaagcccgaggctgagaagacagatcctgaggaaataggcaaagtctcccctttacagatgagagtcctgcactcaggcttggcagtgtgagccgcccattgcaggtgaacagagcctggtctctgtgggatccctgtggggcttgcaggccagcgcctctgctttaaagagaagcctctctccactgcatccctaagcgcttgtgtcgccattgtattcccggaagtgacctttcttctagaagactctagggtgtgacttctgaagagaagaaggaagaggaagggtggaggttaggaaacagtgagtcgggcttgtgggtctctcctggtgatctgacagcttctgggtcagaactcggagtcaccacgacaaactgctctctgtccgcagtacagggttcaggcaaagtcttggttgccaggcggtgaggtcaggggtggggaagcccagggctggggattccccatctcctcagtttcacttctgcacctaacctgggtcaggtccttctgccgggacactgatgacgcgctggcaggtctcactatcattgggtggcgagattccaggagccaatcagcgtcgccgcggacgctggttataaagtccacgcaacccgcgggactcagacacccgggatcccagatgggcgccatggcccctagaaccctgctgctgctcctggccgctgccctggcccctacccagaccagagccattcagagaacaccaaagattcaggtgtactcaaggcacccagccgaaaacggcaagtcaaactttctgaattgctatgtgtctgggtttcatcctagcgatatcgaggtggacctcctcaaaaatggggagaggattgagaaagtggaacactccgatctcagtttcagtaaagattggagtttctatctgctctactataccgaattcacaccaactgaaaaggacgagtacgcctgtagggtcaaccatgtcactctgagccagccaaagattgtgaagtgggatagggacatggggggtggtggcagtggtggtggtggttcaggcggcggtggcagctgctcccactctatgcggtatttcgataccgccgtgtctagaccaggccgcggagaacctagattcatcagcgtcggctatgtggatgacactcagttcgtccgctttgactccgatgctgcctcccctagaggggagcctagggccccttgggtcgagcaggaaggccctgaatattgggacagagagacacagaagtataagcggcaggctcaggcagacagagtgtctctgaggaacctcagaggctactataaccagtccgaggacggatctcacaccctgcagagaatgagcggctgcgatctgggccctgatggacggctgctccgcggctacgaccagagcgcatacgatgggaaggactatatcgcactcaatgaggatctccgctcatggacagctgcagacactgctgcccagatcacacagaggaagctcgaggccgccagagccgctgaacagctgagggcatatctcgaaggcacttgtgtcgagtggctccgccgatacctcgaaaatggcaaagaaactctgcagcgagctgatagcccaaaggcacacgtcacccatcaccctcgctcaaagggcgaagtcactctgaggtgctgggccctcgggttctatcctgccgatatcacactcacctggcagctcaatggcgaggaactgacacaggacatggaactcgtcgaaactagacccgctggggatggcacctttcagaagtgggccagcgtcgtcgtccccctggggaaagaacagaattacacttgtcgcgtgtaccacgaagggctccctgaaccactcacactgagatgggagccacccccttcaactgacagctacatggtcatcgtggctgtcctcggagtcctgggcgccatggcaattatcggagcagtcgtcgccttcgtgatgaagcgacgccggaacacaggtggcaaaggtggcgattatgcactggcaccaggctctcagagtagcgaaatgtcactgagagattgcaaagcctgactgtgccttctagttgccagccatctgttgtttgcccctcccccgtgccttccttgaccctggaaggtgccactcccactgtcctttcctaataaaatgaggaaattgcatcgcattgtctgagtaggtgtcattctattctggggggtggggtggggcaggacagcaagggggaggattgggaagacaatagcaggcatgctggggatgcggtgggctctatggttaattaagcagagaggatatgctcatcgtctaaagaactacccattttattatatattagtcacgatatctataacaagaaaatatatatataataagttatcacgtaagtagaacatgaaataacaatataattatcgtatgagttaaatcttaaaagtcacgtaaaagataatcatgcgtcattttgactcacgcggtcgttatagttcaaaatcagtgacacttaccgcattgacaagcacgcctcacgggagctccaagcggcgactgagatgtcctaaatgcacagcgacggattcgcgctatttagaaagagagagcaatatttcaagaatgcatgcgtcaattttacgcagactatctttctagggttaaaaaagatttgcgctttactcgacctaaactttaaacac

SEQ ID NO: 209 - DNA, 19 bp, Artificial Sequence
  Genotyping primer
accgacagagtggacctgg

SEQ ID NO: 210 - DNA, 24 bp, Artificial Sequence
  Genotyping primer
tcccactttctcttggtgatctgg

SEQ ID NO: 211 - DNA, 22 bp, Artificial Sequence
  Genotyping primer
caaagctcagtcccagacagac

SEQ ID NO: 212 - DNA, 21 bp, Artificial Sequence
  Genotyping primer
ccgctttgtaatctgagcagc

SEQ ID NO: 213 - DNA, 23 bp, Artificial Sequence
  Genotyping primer
cccagatctacaaggctcaggcc

SEQ ID NO: 214 - DNA, 20 bp, Artificial Sequence
  Genotyping primer
taggcccttctctgctcagc

SEQ ID NO: 215 - DNA, 25 bp, Artificial Sequence
  Genotyping primer
caacacccagacatacagagagtcc

SEQ ID NO: 216 - DNA, 22 bp, Artificial Sequence
  Genotyping primer
acgcacagtccttccagatagg

SEQ ID NO: 217 - DNA, 23 bp, Artificial Sequence
  Genotyping primer
cccagaagtacaagagacaggcc

SEQ ID NO: 218 - DNA, 20 bp, Artificial Sequence
  Genotyping primer
gataggctctgcgctgttcg

SEQ ID NO: 219 - DNA, 23 bp, Artificial Sequence
  Genotyping primer
gaacctagattcatcagcgtcgg

SEQ ID NO: 220 - DNA, 25 bp, Artificial Sequence
  Genotyping primer
cggactggttatagtagcctctgag

SEQ ID NO: 221 - DNA, 23 bp, Artificial Sequence
  Genotyping primer
ggccgttcttagttggtggagcg

SEQ ID NO: 222 - DNA, 20 bp, Artificial Sequence
  Genotyping primer
ctgaacgccacttgtccctc

SEQ ID NO: 223 - DNA, 20 bp, Artificial Sequence
  Genotyping primer
atggcaaaaaccaagtggag

SEQ ID NO: 224 - DNA, 20 bp, Artificial Sequence
  Genotyping primer
cacattaggccaggagaagc

SEQ ID NO: 225 - DNA, 20 bp, Artificial Sequence
  Genotyping primer
tttgctttgtgtctgcatcc

SEQ ID NO: 226 - DNA, 20 bp, Artificial Sequence
  Genotyping primer
cctgcttagtggctgagtgg

SEQ ID NO: 227 - DNA, 728 bp, Artificial Sequence
  H-2Db promoter
cgcgccttcttctacataaaacacacccatctggagctacagaggcttcatatgggaagaaacaggaggagtctgagactaagcccgaggctgagaagacagatcctgaggaaataggcaaagtctcccctttacagatgagagtcctgcactcaggcttggcagtgtgagccgcccattgcaggtgaacagagcctggtctctgtgggatccctgtggggcttgcaggccagcgcctctgctttaaagagaagcctctctccactgcatccctaagcgcttgtgtcgccattgtattcccggaagtgacctttcttctagaagactctagggtgtgacttctgaagagaagaaggaagaggaagggtggaggttaggaaacagtgagtcgggcttgtgggtctctcctggtgatctgacagcttctgggtcagaactcggagtcaccacgacaaactgctctctgtccgcagtacagggttcaggcaaagtcttggttgccaggcggtgaggtcaggggtggggaagcccagggctggggattccccatctcctcagtttcacttctgcacctaacctgggtcaggtccttctgccgggacactgatgacgcgctggcaggtctcactatcattgggtggcgagattccaggagccaatcagcgtcgccgcggacgctggttataaagtccacgcaacccgcgggactcagacacccgggatcccag

SEQ ID NO: 228 - DNA, 225 bp, Artificial Sequence
  bovine growth hormone (bGH) polyadenylation signal
ctgtgccttctagttgccagccatctgttgtttgcccctcccccgtgccttccttgaccctggaaggtgccactcccactgtcctttcctaataaaatgaggaaattgcatcgcattgtctgagtaggtgtcattctattctggggggtggggtggggcaggacagcaagggggaggattgggaagacaatagcaggcatgctggggatgcggtgggctctatgg

SEQ ID NO: 229 - DNA, 57 bp, Artificial Sequence
  2A peptide linker
ctgtgccttctagttgccagccatctgttgtttgcccctcccccgtgccttccttga

SEQ ID NO: 230 - DNA, 72 bp, Artificial Sequence
  Leader sequence
atgggcgccatggcccctagaaccctgctgctgctcctggccgctgccctggcccctacccagaccagagcc

SEQ ID NO: 231 - DNA, 235 bp, Artificial Sequence
  5'-PiggyBac-ITR
ttaaccctagaaagataatcatattgtgacgtacgttaaagataatcatgcgtaaaattgacgcatgtgttttatcggtctgtatatcgaggtttatttattaatttgaatagatattaagttttattatatttacacttacatactaataataaattcaacaaacaatttatttatgtttatttatttattaaaaaaaaacaaaaactcaaaatttcttctataaagtaacaaa

SEQ ID NO: 232 - DNA, 313 bp, Artificial Sequence
  3'-PiggyBac-ITR
gatatctataacaagaaaatatatatataataagttatcacgtaagtagaacatgaaataacaatataattatcgtatgagttaaatcttaaaagtcacgtaaaagataatcatgcgtcattttgactcacgcggtcgttatagttcaaaatcagtgacacttaccgcattgacaagcacgcctcacgggagctccaagcggcgactgagatgtcctaaatgcacagcgacggattcgcgctatttagaaagagagagcaatatttcaagaatgcatgcgtcaattttacgcagactatctttctagggttaa

SEQ ID NO: 233 - DNA, 297 bp, Artificial Sequence
  ß2-microglobulin leader sequence
atccagcgcactcctaagattcaggtctacagccgccacccagctgaaaacggaaagtccaatttcctcaactgctatgtctctggatttcacccctccgacattgaagtggacctgctcaaaaatggcgaacgcattgagaaagtcgagcatagcgatctcagcttctccaaggattggtctttttatctgctctattacacagaattcacccctacagaaaaggatgaatacgcatgtcgagtgaatcacgtcacactctcccagccaaaaattgtgaagtgggaccgcgatatg